European Patent Application EP 4 656 207 A1, published December 3, 2025. Title: IN VITRO METHOD FOR TRANSDUCING A TARGET CELL. Applicant: FUNDACIÓ HOSPITAL UNIVERSITARI VALL D'HEBRON - INSTITUT DE RECERCA. The sequence listing filed with the application follows.

SEQUENCE LISTING (17 sequences)

SEQ ID NO: 1 - protein, 9 aa, synthetic construct
IKVKLEAEI

SEQ ID NO: 2 - protein, 8 aa, synthetic construct
ATYRRLLE

SEQ ID NO: 3 - protein, 20 aa, synthetic construct
LLNIKVKLEAEIATYRRLLE

SEQ ID NO: 4 - protein, 9 aa, synthetic construct
CRGDKGPDC

SEQ ID NO: 5 - protein, 8 aa, synthetic construct
KKKKKKKK

SEQ ID NO: 6 - protein, 8 aa, synthetic construct
RRRRRRRR

SEQ ID NO: 7 - protein, 6 aa, synthetic construct
HHHHHH

SEQ ID NO: 8 - protein, 20 aa, synthetic construct
LLNIKVKLEAEIRRRRRRRR

SEQ ID NO: 9 - protein, 20 aa, synthetic construct
LLNVKMALDIEIRRRRRRRR

SEQ ID NO: 10 - protein, 21 aa, synthetic construct
LLNKEIKIEVALARRRRRRRR

SEQ ID NO: 11 - protein, 9 aa, synthetic construct
VKMALDIEI

SEQ ID NO: 12 - DNA, 21 bp, synthetic construct
  source 1..21: mol_type = other DNA
gctgtcatctcttgtgggctg

SEQ ID NO: 13 - DNA, 21 bp, synthetic construct
  source 1..21: mol_type = other DNA
actcatgggagctgctggttc

SEQ ID NO: 14 - DNA, 20 bp, synthetic construct
  source 1..20: mol_type = other DNA
caggactcggcttgctgaag

SEQ ID NO: 15 - DNA, 20 bp, synthetic construct
  source 1..20: mol_type = other DNA
tcccccgcttaatactgacg

SEQ ID NO: 16 - DNA, 26 bp, synthetic construct
  source 1..26: mol_type = other DNA
cctgtcatgcccacacaaatctctcc

SEQ ID NO: 17 - DNA, 19 bp, synthetic construct
  source 1..19: mol_type = other DNA
cgcacggcaagaggcgagg